European Patent Specification EP 4 153 779 B1, published February 25, 2026. Title: FLUORESCENT POLYNUCLEOTIDE SEQUENCING METHODS AND COMPOSITIONS. Applicant: QUANTAPORE, INC. SIMONS, Jan F. HUBER, Martin. Application EP21791708.7. The sequence listing filed with the application follows.

SEQUENCE LISTING (8 sequences)

SEQ ID NO: 1 - DNA, 22 bp, Artificial Sequence
  random sequence
actgggttccagttaccctgga

SEQ ID NO: 2 - DNA, 22 bp, Artificial Sequence
  random sequence
tccagggtaactggaacccagt

SEQ ID NO: 3 - DNA, 20 bp, Artificial Sequence
  random sequence
gctatgtggcgcggtattat

SEQ ID NO: 4 - DNA, 20 bp, Artificial Sequence
  random sequence
gctatgtggcgcggtattag

SEQ ID NO: 5 - DNA, 200 bp, Artificial Sequence
  random sequence
gactactaggtctctagacgctggatcttccaaattaacacccacccaggtagctagagtcattagttccccccagcaaagaattgcttgcctgagtgcagtatggtgaggtgaacaatgctcaggagactctaaggcttcccgatacagagctgaggcggtatctagaagatctcgtacctaataccgcgccacatagc

SEQ ID NO: 6 - DNA, 180 bp, Artificial Sequence
  random sequence
guacgagaucuucuagauaccgccucagcucuguaucgggaagccuuagagucuccugagcauuguucaccucaccauacugcacucaggcaagcaauucuuugcuggggggaacuaaugacucuagcuaccuggguggguguuaauuuggaagauccagcgucuagagaccuaguaguc

SEQ ID NO: 7 - DNA, 20 bp, Artificial Sequence
  random sequence
actgggttccagttaccctg

SEQ ID NO: 8 - DNA, 21 bp, Artificial Sequence
  random sequence
actgggttccagttaccctgg